European Patent Specification EP 3 833 738 B1, published June 25, 2025. Title: PROBIOTIC BACTERIA ISOLATED FROM WOLVES AND RELATED COMPOSITIONS AND METHODS. Applicant: CanBiocin Inc. The sequence listing filed with the application follows.

SEQUENCE LISTING (28 sequences)

SEQ ID NO: 1 - DNA, 767 bp, Lactobacillus reuteri
  misc_feature (456)..(456): n is a, t, g, or c
  misc_feature (561)..(561): r is a or g
agcgtcagttgcagaccagacagccgccttcgccactggtgttcttccatatatctacgcattccaccgctacacatggagttccactgtcctcttctgcactcaagtcgcccggtttccgatgcacttcttcggttaagccgaaggctttcacatcagacctaagcaaccgcctgcgctcgctttacgcccaataaatccggataacgcttgccacctacgtattaccgcggctgctggcacgtagttagccgtgactttctggttggataccgtcactgcgtgaacagttactctcacgcacgttcttctccaacaacagagctttacgagccgaaacccttcttcactcacgcggtgttgctccatcaggcttgcgcccattgtggaagattccctactgctgcctcccgtaggagtatggaccgtgtctcagttccattgtggccgatcagnctctcaactcggctatgcatcatcgccttggtaagccgttaccttaccaactagctaatgcaccgcaggtccatcccagagtgatagccaaagccatctttcaarcaaaagccatgtggcttttgttgttatgcggtattagcatctgtttccaaatgttatcccccgctccggggcaggttacctacgtgttactcacccgtccgccactcactggtgatccatcgtcaatcaggtgcaagcaccatcaatcagttgggccagtgcgtacgacttgcatgtattaggcacaccgccggcgttcatcctga

SEQ ID NO: 2 - DNA, 692 bp, Lactobacillus animalis
ttacagaccagagagccgctttcgccactggtgttcttccatatatctacgcatttcaccgctacacatggagttccactctcctcttctgcactcaagtctcccagtttccaatgcactactccggttaagccgaaggctttcacatcagacttaaaagaccgcctgcgttccctttacgcccaataaatccggataacgcttgccacctacgtattaccgcggctgctggcacgtagttagccgtggctttctggttagataccgtcgaaacgtgaacagttactctcacgcactttcttctctaacaacagggttttacgatccgaagaccttcttcacccacgcggcgttgctccatcaggctttcgcccattgtggaagattccctactgctgcctcccgtaggagtttgggccgtgtctcagtcccaatgtggccgatcaacctctcagttcggctacgcatcattgccttggtaagcctttacctcaccaactagctaatgcgccgcgggcccatccaaaagcggtagcatagccaccttttacatagttaccatgcggtaactatggttatgcggtattagcacctgtttccaagtgttatccccctcttttgggcaggttgcccacgtgttactcacccgttcgccactcaactctttatcggtgagtgcaagcactcggtga

SEQ ID NO: 3 - DNA, 706 bp, Enterococcus faecium
  misc_feature (558)..(558): n is a, t, g, or c
agccgccttcgccactggtgttcctccatatatctacgcatttcaccgctacacatggaattccactctcctcttctgcactcaagtctcccagtttccaatgaccctccccggttgagccgggggctttcacatcagacttaagaaaccgcctgcgctcgctttacgcccaataaatccggacaacgcttgccacctacgtattaccgcggctgctggcacgtagttagccgtggctttctggttagataccgtcaagggatgaacagttactctcatccttgttcttctctaacaacagagttttacgatccgaaaaccttcttcactcacgcggcgttgctcggtcagactttcgtccattgccgaagattccctactgctgcctcccgtaggagtttgggccgtgtctcagtcccaatgtggccgatcaccctctcaggtcggctatgcatcgtggccttggtgagccgttacctcaccaactagctaatgcaccgcgggtccatccatcagcgacacccgaaagcgcctttcaaatcaaaaccatgcggtttngattgttatacggtattagcacctgtttccaagtgttatccccttctgatgggcaggttacccacgtgttactcacccgttcgccactcctctttttccggtggagcaagctccggtggaaaaagaagcgttcgacttgcatgtatta

SEQ ID NO: 4 - DNA, 760 bp, Lactobacillus plantarum
  misc_feature (109)..(109): y is c or t
  misc_feature (146)..(146): n is a, t, g, or c
  misc_feature (561)..(561): n is a, t, g, or c
  misc_feature (734)..(734): n is a, t, g, or c
agcgtcagttacagaccagacagccgccttcgccactggtgttcttccatatatctacgcatttcaccgctacacatggagttccactgtcctcttctgcactcaagtytcccagtttccgatgcacttcttcggttgagccgaangctttcacatcagacttaaaaaaccgcctgcgctcgctttacgcccaataaatccggacaacgcttgccacctacgtattaccgcggctgctggcacgtagttagccgtggctttctggttaaataccgtcaatacctgaacagttactctcagatatgttcttctttaacaacagagttttacgagccgaaacccttcttcactcacgcggcgttgctccatcagactttcgtccattgtggaagattccctactgctgcctcccgtaggagtttgggccgtgtctcagtcccaatgtggccgattaccctctcaggtcggctacgtatcattgccatggtgagccgttaccccaccatctagctaatacgccgcgggaccatccaaaagtgatagccgaagccatctttcaanctcggaccatgcggtccaagttgttatgcggtattagcatctgtttccaggtgttatcccccgcttctgggcaggtttcccacgtgttactcaccagttcgccactcactcaaatgtaaatcatgatgcaagcaccaatcaataccagagttcgttcgacttgcatgtattangcacgccgccagcgttcgtcctgagc

SEQ ID NO: 5 - DNA, 739 bp, Lactobacillus brevis
  misc_feature (560)..(560): n is a, t, g, or c
  misc_feature (715)..(715): n is a, t, g, or c
acagccgccttcgccactggtgttcttccatatatctacgcattccaccgctacacatggagttccactgtcctcttctgcactcaagtctcccagtttccgatgcacttctccggttaagccgaaggctttcacatcagacttaaaaaaccgcctgcgctcgctttacgcccaataaatccggacaacgcttgccacctacgtattaccgcggctgctggcacgtagttagccgtggctttctggttaaataccgtcaacccttgaacagttactctcaaaggtgttcttctttaacaacagagttttacgagccgaaacccttcttcactcacgcggcattgctccatcagactttcgtccattgtggaagattccctactgctgcctcccgtaggagtttgggccgtgtctcagtcccaatgtggccgattaccctctcaggtcggctacgtatcatcgtcttggtgggcctttacctcaccaactaactaatacgccgcgggatcatccagaagtgatagccgaagccacctttcaaacaaaatccatgcggattntgttgttatacggtattagcacctgtttccaagtgttatcccctgcttctgggcagatttcccacgtgttactcaccagttcgccactcgcttcattgttgaaatcagtgcaagcacgtcattcaacggaagctcgttcgacttgcatgtattangcatgccgccagcgttcgtcctga

SEQ ID NO: 6 - DNA, 765 bp, Lactobacillus curvatus
  misc_feature (737)..(737): n is a, t, g, or c
gcgtcagttacagaccagacagccgccttcgccactggtgttcttccatatatctacgcatttcaccgctacacatggagttccactgtcctcttctgcactcaagtttcccagtttccgatgcacttcttcggttgagccgaaggctttcacatcagacttaagaaaccgcctgcgctcgctttacgcccaataaatccggacaacgcttgccacctacgtattaccgcggctgctggcacgtagttagccgtggctttctggttggataccgtcactacctgatcagttactatcaaatacgttcttctccaacaacagagttttacgatccgaaaaccttcttcactcacgcggcgttgctccatcagactttcgtccattgtggaagattccctactgctgcctcccgtaggagtctgggccgtgtctcagtcccagtgtggccgattaccctctcaggtcggctatgcatcacggtcttggtgagcctttacctcaccaactaactaatgcaccgcgggtccatcctaaagtgatagccgaaaccatctttcaaccttgcaccatgcggtgctaggttttatgcggtattagcatctgtttccaaatgttatcccccactttagggcaggttacccacgtgttactcacccgtccgccactcactcaaatgttatcaatcagaagcaagcttcttcaatctaacgagagtgcgttcgacttgcatgtattangcacgccgccagcgttcgtcctgagcca

SEQ ID NO: 7 - DNA, 767 bp, Lactobacillus reuteri
  misc_feature (166)..(166): n is a, t, g, or c
  misc_feature (456)..(456): n is a, t, g, or c
  misc_feature (561)..(561): n is a, t, g, or c
  misc_feature (635)..(635): n is a, t, g, or c
  misc_feature (728)..(728): n is a, t, g, or c
agcgtcagttgcagaccagacagccgccttcgccactggtgttcttccatatatctacgcattccaccgctacacatggagttccactgtcctcttctgcactcaagtcgcccggtttccgatgcacttcttcggttaagccgaaggctttcacatcagacctaancaaccgcctgcgctcgctttacgcccaataaatccggataacgcttgccacctacgtattaccgcggctgctggcacgtagttagccgtgactttctggttggataccgtcactgcgtgaacagttactctcacgcacgttcttctccaacaacagagctttacgagccgaaacccttcttcactcacgcggtgttgctccatcaggcttgcgcccattgtggaagattccctactgctgcctcccgtaggagtatggaccgtgtctcagttccattgtggccgatcagnctctcaactcggctatgcatcatcgccttggtaagccgttaccttaccaactagctaatgcaccgcaggtccatcccagagtgatagccaaagccatctttcaancaaaagccatgtggcttttgttgttatgcggtattagcatctgtttccaaatgttatcccccgctccggggcangttacctacgtgttactcacccgtccgccactcactggtgatccatcgtcaatcaggtgcaagcaccatcaatcagttgggccagtgcgtacnacttgcatgtattaggcacaccgccggcgttcatcctga

SEQ ID NO: 8 - DNA, 20 bp, Artificial Sequence
  Synthetic Primer
agagtttgatcctggctcag

SEQ ID NO: 9 - DNA, 20 bp, Artificial Sequence
  Synthetic Primer
gactaccagggtatctaatc

SEQ ID NO: 10 - DNA, 15 bp, Artificial Sequence
  Synthetic primer
gagggtggcggttct

SEQ ID NO: 11 - DNA, 20 bp, Artificial Sequence
  Synthetic Primer
ctcaccagcacctttgtcca

SEQ ID NO: 12 - DNA, 20 bp, Artificial Sequence
  Synthetic Primer
ctccttgtccgtcaccaacc

SEQ ID NO: 13 - DNA, 20 bp, Artificial Sequence
  Synthetic Primer
gcactgagaaaggaggtggg

SEQ ID NO: 14 - DNA, 20 bp, Artificial Sequence
  Synthetic Primer
cctgagaccagcagcagaaa

SEQ ID NO: 15 - DNA, 20 bp, Artificial Sequence
  Synthetic Primer
aacccctcccttctcaaact

SEQ ID NO: 16 - DNA, 20 bp, Artificial Sequence
  Synthetic Primer
tagaacccacaactgctggc

SEQ ID NO: 17 - DNA, 18 bp, Artificial Sequence
  Synthetic Primer
ggggaaaggatgccccaa

SEQ ID NO: 18 - DNA, 20 bp, Artificial Sequence
  Synthetic Primer
acggagctgtggttaatggg

SEQ ID NO: 19 - DNA, 20 bp, Artificial Sequence
  Synthetic Primer
cctgactggtggatgtgacc

SEQ ID NO: 20 - DNA, 21 bp, Artificial Sequence
  Synthetic Primer
gcagtcctggtaaatgtggga

SEQ ID NO: 21 - DNA, 20 bp, Artificial Sequence
  Synthetic Primer
catctccttctgctgctggt

SEQ ID NO: 22 - DNA, 20 bp, Artificial Sequence
  Synthetic Primer
acaagaatggcacagagggg

SEQ ID NO: 23 - DNA, 20 bp, Artificial Sequence
  Synthetic Primer
tcattcgtttcctcccaccg

SEQ ID NO: 24 - DNA, 20 bp, Artificial Sequence
  Synthetic Primer
atctctctgggctctggctt

SEQ ID NO: 25 - DNA, 21 bp, Artificial Sequence
  Synthetic Primer
gccagtagctcatgttgtagg

SEQ ID NO: 26 - DNA, 16 bp, Artificial Sequence
  Synthetic Primer
tggccctcgggttctg

SEQ ID NO: 27 - DNA, 20 bp, Artificial Sequence
  Synthetic Primer
ggattaagttggggcaggga

SEQ ID NO: 28 - DNA, 20 bp, Artificial Sequence
  Synthetic Primer
aaagcagttgggagtctggc